European Patent Application EP 4 155 399 A1, published March 29, 2023. Title: ACETOLACTATE DECARBOXYLASE. Applicant: DuPont Nutrition Biosciences ApS. The sequence listing filed with the application follows.

SEQUENCE LISTING (8 sequences)

SEQ ID NO: 1 - DNA, 858 bp, Brevibacillus brevis
  source 1..858: mol_type = genomic DNA
atgaaaaaaaatatcatcacttctatcacatctctggctctggttgccgggctgtctttgactgcttttgcagctacaacggctactgtaccagcaccacctgccaagcaggaatccaaacctgcggttgccgctaatccggcaccaaaaaatgtactgtttcaatactcaacgatcaatgcactcatgcttggacagtttgaaggggacttgactttgaaagacctgaagctgcgaggcgatatggggcttggtaccatcaatgatctcgatggagagatgattcagatgggtacaaaattctaccagatcgacagcaccggaaaattatcggagctgccagaaagtgtgaaaactccatttgcggttactacacatttcgagccgaaagaaaaaactacattaaccaatgtgcaagattacaatcaattaacaaaaatgcttgaggagaaatttgaaaacaagaacgtcttttatgccgtaaagctgaccggtacctttaagatggtaaaggctagaacagttccaaaacaaaccagaccttatccgcagctgactgaagtaaccaaaaaacaatccgagtttgaatttaaaaatgttaagggaaccctgattggcttctatacgccaaattatgcagcagccctgaatgttcccggattccatctccacttcatcacagaggataaaacaagtggcggacacgtattaaatctgcaatttgacaacgcgaatctggaaatttctccgatccatgagtttgatgtacaattgccgcacacagatgattttgcccactctgatctgacacaagttactactagccaagtacaccaagctgagtcagaaagaaaataa

SEQ ID NO: 2 - protein, 285 aa, Brevibacillus brevis
MKKNIITSITSLALVAGLSLTAFAATTATVPAPPAKQESKPAVAANPAPKNVLFQYSTINALMLGQFEGDLTLKDLKLRGDMGLGTINDLDGEMIQMGTKFYQIDSTGKLSELPESVKTPFAVTTHFEPKEKTTLTNVQDYNQLTKMLEEKFENKNVFYAVKLTGTFKMVKARTVPKQTRPYPQLTEVTKKQSEFEFKNVKGTLIGFYTPNYAAALNVPGFHLHFITEDKTSGGHVLNLQFDNANLEISPIHEFDVQLPHTDDFAHSDLTQVTTSQVHQAESERK

SEQ ID NO: 3 - protein, 261 aa, Brevibacillus brevis
ATTATVPAPPAKQESKPAVAANPAPKNVLFQYSTINALMLGQFEGDLTLKDLKLRGDMGLGTINDLDGEMIQMGTKFYQIDSTGKLSELPESVKTPFAVTTHFEPKEKTTLTNVQDYNQLTKMLEEKFENKNVFYAVKLTGTFKMVKARTVPKQTRPYPQLTEVTKKQSEFEFKNVKGTLIGFYTPNYAAALNVPGFHLHFITEDKTSGGHVLNLQFDNANLEISPIHEFDVQLPHTDDFAHSDLTQVTTSQVHQAESERK

SEQ ID NO: 4 - DNA, 783 bp, synthetic construct
  misc_feature 1..783: note = mature sequence of the aldB gene in plasmid RIHI-aldB
  source 1..783: mol_type = other DNA
gctacaacggctactgtaccagcaccacctgccaagcaggaatccaaacctgcggttgccgctaatccggcaccaaaaaatgtactgtttcaatactcaacgatcaatgcactcatgcttggacagtttgaaggggacttgactttgaaagacctgaagctgcgaggcgatatggggcttggtaccatcaatgatctcgatggagagatgattcagatgggtacaaaattctaccagatcgacagcaccggaaaattatcggagctgccagaaagtgtgaaaactccatttgcggttactacacatttcgagccgaaagaaaaaactacattaaccaatgtgcaagattacaatcaattaacaaaaatgcttgaggagaaatttgaaaacaagaacgtcttttatgccgtaaagctgaccggtacttttaagatggtaaaggctagaacagttccaaaacaaaccagaccttatccgcagctgactgaagtaaccaaaaaacaatccgagtttgaatttaaaaatgttaagggaaccctgattggcttctatacgccaaattatgcagcagccctgaatgttcccggattccatctccacttcatcacagaggataaaacaagtggcggacacgtattaaatctgcaatttgacaacgcgaatctggaaatttctccgatccatgagtttgatgttcaattgccgcacacagatgattttgcccactctgatctgacacaagttactactagccaagtacaccaagctgagtcagaaagaaaa

SEQ ID NO: 5 - protein, 290 aa, synthetic construct
  REGION 1..290: note = aldB precursor protein expressed from plasmid RIHI-aldB
VRSKKLWISLLFALTLIFTMAFSNMSAQAATTATVPAPPAKQESKPAVAANPAPKNVLFQYSTINALMLGQFEGDLTLKDLKLRGDMGLGTINDLDGEMIQMGTKFYQIDSTGKLSELPESVKTPFAVTTHFEPKEKTTLTNVQDYNQLTKMLEEKFENKNVFYAVKLTGTFKMVKARTVPKQTRPYPQLTEVTKKQSEFEFKNVKGTLIGFYTPNYAAALNVPGFHLHFITEDKTSGGHVLNLQFDNANLEISPIHEFDVQLPHTDDFAHSDLTQVTTSQVHQAESERK

SEQ ID NO: 6 - DNA, 858 bp, synthetic construct
  misc_feature 1..858: note = sequence encoding an acetolactate decarboxylase
  source 1..858: mol_type = other DNA
atgaaaaaaaatatcatcacttctatcacatctctggctctcgttgccgggctgtctttgactgcttttgcagctacaacggctactgtaccagcaccacctgccaagcaggaatccaaacctgtggttgccgctaatccggcaccaaaaaatgtactgtttcaatactcaacgatcaatgcactcatgcttggacagtttgaaggggacttgactttgaaagacctgaagctacgaggcgatatggggcttggtaccatcaatgatctcgatggagagatgattcagatgggtacaaaattctaccagatcgacagcaccggaaaattatccgagctgccagaaagtgtgaaaactccatttgcggttactacacatttcgagccgaaagaaaaaactacattaaccaatgtgcaagattacaatcaattaacaaaaatgcttgaggagaaatttgaaaacaagaacgtcttttatgccgtaaagctgaccggtacctttaagatggtaaaggctagaacagttccaaaacaaaccagaccttatccgcagctgactgaagtaaccaaaaaacaatccgagtttgaatttaaaaatgttaagggaaccctgattggcttctatacgccaaattatgcagcagccctgaatgttcccggattccatctccacttcatcacagaggataaaacaagtggcggacacgtattaaatctgcaatttgacaacgcgaatctggaaatttctccgatccatgagtttgatgtacaattgccgcacacagatgattttgcccactctgatctgacacaagttactactagccaagtacaccaagctgagtcagaaagaaaataa

SEQ ID NO: 7 - protein, 285 aa, synthetic construct
  REGION 1..285: note = sequence of acetolactate decarboxylase (ALDC) precursor aldB
MKKNIITSITSLALVAGLSLTAFAATTATVPAPPAKQESKPVVAANPAPKNVLFQYSTINALMLGQFEGDLTLKDLKLRGDMGLGTINDLDGEMIQMGTKFYQIDSTGKLSELPESVKTPFAVTTHFEPKEKTTLTNVQDYNQLTKMLEEKFENKNVFYAVKLTGTFKMVKARTVPKQTRPYPQLTEVTKKQSEFEFKNVKGTLIGFYTPNYAAALNVPGFHLHFITEDKTSGGHVLNLQFDNANLEISPIHEFDVQLPHTDDFAHSDLTQVTTSQVHQAESERK

SEQ ID NO: 8 - protein, 261 aa, synthetic construct
  REGION 1..261: note = predicted amino acid sequence of the mature acetolactatedecarboxylase (ALDC) aldB
ATTATVPAPPAKQESKPVVAANPAPKNVLFQYSTINALMLGQFEGDLTLKDLKLRGDMGLGTINDLDGEMIQMGTKFYQIDSTGKLSELPESVKTPFAVTTHFEPKEKTTLTNVQDYNQLTKMLEEKFENKNVFYAVKLTGTFKMVKARTVPKQTRPYPQLTEVTKKQSEFEFKNVKGTLIGFYTPNYAAALNVPGFHLHFITEDKTSGGHVLNLQFDNANLEISPIHEFDVQLPHTDDFAHSDLTQVTTSQVHQAESERK